European Patent Application EP 4 282 968 A1, published November 29, 2023. Title: Gene Transcription Framework, Vector System, Genome Sequence Editing Method and Application. Applicant: Peng, Shuanghong. Application EP21920753.7. The sequence listing filed with the application follows.

SEQUENCE LISTING (54 sequences)

SEQ ID NO: 1 - DNA, 333 bp, Artificial sequence
  The complete sequence of the Alu element (sequence).
gggccgggcgcggtggctcacgcctgtaatcccagcactttgggaggccgaggcgggcggatcacgaggtcaggagatcgagaccatcccggctaaaacggtgaaaccccgtctctactaaaaatacaaaaaattagccgggcgtggtggcgggcgcctgtagtcccagctactcgggaggctgaggcaggagaatggcgtgaacccgggaggcggagcttgcagtgagccgagatcacgccgctgcactccaccctgggcgacagagcgagactccgtctcaaaaaaaaaaaaaaaaaaaaaaaaaaaaaagattaataactgctggagatc

SEQ ID NO: 2 - DNA, 217 bp, Artificial sequence
  The partial Alu sequence.
actaaaaatacaaaaaattagccgggcgtggtggcgggcgcctgtagtcccagctactcgggaggctgaggcaggagaatggcgtgaacccgggaggcggagcttgcagtgagccgagatcacgccgctgcactccaccctgggcgacagagcgagactccgtctcaaaaaaaaaaaaaaaaaaaaaaaaaaaaaagattaataactgctggagatc

SEQ ID NO: 3 - DNA, 459 bp, Artificial sequence
  A 459-bp selected sequence of the gene VEGFA in the human genome.
attatgcggatcaaacctcaccaaggccagcacataggagagatgagcttcctacagcacaacaaatgtgaatgcaggtgaggatgtagtcacggattcattatcagcaagtggctgcagggtgcctgatctgtgccagggttaagcatgctgtactttttggcccccgtccagcttcccgctatgtgacctttggcattttacttcaatgtgcctcagtttctacatctgtaaaatgggcacaatagtagtatacttcatagcattgttataatgattaaacaagttatatatgaaaagattaaaacagtgttgctccataataaatgctgtttttactgtgattattattgttgttatccctatcattatcatcaccatcttaacccttccctgttttgctcttttctctctccctacccattgcagaccaaagaaagatagagcaagacaagaaaa

SEQ ID NO: 4 - DNA, 521 bp, Artificial sequence
  The Seq ID No.3 with the sequence to be inserted and NheI enzyme cutting sites and protective bases.
ctagctagctagattatgcggatcaaacctcaccaaggccagcacataggagagatgagcttcctacagcacaacaaatgtgaatgcaggtgaggatgtagtcacggattcattatcagcaagtggctgcagggtgcctgatctgtgccagggttaagcatgctgtactttttggcccccgtccagcttcccgctatgtgacctttggcattttacttcaatgtgcctcagtttctacatctgtaaaatgggcacgctacggaataagaggaggccacaacagtcgtgggtcgaatagtagtatacttcatagcattgttataatgattaaacaagttatatatgaaaagattaaaacagtgttgctccataataaatgctgtttttactgtgattattattgttgttatccctatcattatcatcaccatcttaacccttccctgttttgctcttttctctctccctacccattgcagaccaaagaaagatagagcaagacaagaaaactagctagctag

SEQ ID NO: 5 - DNA, 82 bp, Artificial sequence
  The Seq ID No.4 with shorter upstream sequence of target site and downstream sequence of target site.
ctagctagctagaaatgggcacgctacggaataagaggaggccacaacagtcgtgggtcgaatagtagtactagctagctag

SEQ ID NO: 6 - DNA, 456 bp, Artificial sequence
  Alu sequence with non-homologous sequence, “TTTTT” sequence, “TTTTAA” sequence, and SalI enzyme cutting site and corresponding protective base.
acgcgtcgacgtcggccatagcggccgcggaagggccgggcgcggtggctcacgcctgtaatcccagcactttgggaggccgaggcgggcggatcacgaggtcaggagatcgagaccatcccggctaaaacggtgaaaccccgtctctactaaaaatacaaaaaattagccgggcgtggtggcgggcgcctgtagtcccagctactcgggaggctgaggcaggagaatggcgtgaacccgggaggcggagcttgcagtgagccgagatcacgccgctgcactccaccctgggcgacagagcgagactccgtctcaaaaaaaaaaaaaaaaaaaaaaaaaaaaaagattaataactgctggagatcctatcaggcgagcccgtatttttttttaattttaattttaattttaattttaattttaaacgcgtcgacgtcggccatagcggccgcggaa

SEQ ID NO: 7 - DNA, 20 bp, Artificial sequence
  The upstream primer sequence for detecting the GAPDH gene.
cactgccacccagaagactg

SEQ ID NO: 8 - DNA, 20 bp, Artificial sequence
  The downstream primer sequence for detecting the GAPDH gene.
cctgcttcaccaccttcttg

SEQ ID NO: 9 - DNA, 18 bp, Artificial sequence
  The upstream primer sequence for detecting the inserted sequence in example 1.
cccagggttgtcccatct

SEQ ID NO: 10 - DNA, 19 bp, Artificial sequence
  The downstream primer sequence for detecting the inserted sequence in example 1.
cctcctcttattccgtagc

SEQ ID NO: 11 - DNA, 18 bp, Artificial sequence
  Another upstream primer sequence for detecting the inserted sequence in example 1.
cacaacagtcgtgggtcg

SEQ ID NO: 12 - DNA, 22 bp, Artificial sequence
  Another downstream primer sequence for detecting the inserted sequence in example 1.
gagggagaagtgctaaagtcag

SEQ ID NO: 13 - DNA, 18 bp, Artificial sequence
  The downstream primer sequence for detecting the connection in example 2.
tacgggctcgcctgatag

SEQ ID NO: 14 - DNA, 479 bp, Artificial sequence
  The 479-bp selected sequence of the gene MMP2 in the human genome.
agcatggcgatggatacccctttgacggtaaggacggactcctggctcatgccttcgccccaggcactggtgttgggggagactcccattttgatgacgatgagctatggaccttgggagaaggccaaggtgagaaaggggccctctgcatgccccagaccttctctcctgtcctctctccactccatttgcttggaccagagaggtgggaggggaggaaagtcacacatctgggtgagtcagaatcttggtctccaaagaaggcctggagaagtccaacctcccccttccatgtcactctttagtggtccgtgtgaagtatgggaacgccgatggggagtactgcaagttccccttcttgttcaatggcaaggagtacaacagctgcactgataccggccgcagcgatggcttcctctggtgctccaccacctacaactttgagaaggatggcaagtacggcttctgtccccatgaag

SEQ ID NO: 15 - DNA, 606 bp, Artificial sequence
  The Seq ID No.14 with the sequence to be inserted and NheI enzyme cutting sites and protective bases.
ctagctagctagagcatggcgatggatacccctttgacggtaaggacggactcctggctcatgccttcgccccaggcactggtgttgggggagactcccattttgatgacgatgagctatggaccttgggagaaggccaaggtgagaaaggggccctctgcatgccccagaccttctctcctgtcctctctccactccatttgcttggaccagagagcctgtgggccttgctcagagcggagaaagcatggcataatgatgtggctgttttgtttgtacaagatccgcagacgtgtaaatgttcctgcaaaaacacagacgtgggaggggaggaaagtcacacatctgggtgagtcagaatcttggtctccaaagaaggcctggagaagtccaacctcccccttccatgtcactctttagtggtccgtgtgaagtatgggaacgccgatggggagtactgcaagttccccttcttgttcaatggcaaggagtacaacagctgcactgataccggccgcagcgatggcttcctctggtgctccaccacctacaactttgagaaggatggcaagtacggcttctgtccccatgaagctagctagctag

SEQ ID NO: 16 - DNA, 147 bp, Artificial sequence
  The Seq ID No.15 with shorter upstream sequence of target site and downstream sequence of target site.
ctagctagctaggaccagagagcctgtgggccttgctcagagcggagaaagcatggcataatgatgtggctgttttgtttgtacaagatccgcagacgtgtaaatgttcctgcaaaaacacagacgtgggaggggctagctagctag

SEQ ID NO: 17 - DNA, 456 bp, Artificial sequence
  Alu sequence with non-homologous sequence, “TTTTT” sequence, “TTTTAA” sequence, and SalI enzyme cutting site and corresponding protective base.
acgcgtcgacgtcggccatagcggccgcggaagggccgggcgcggtggctcacgcctgtaatcccagcactttgggaggccgaggcgggcggatcacgaggtcaggagatcgagaccatcccggctaaaacggtgaaaccccgtctctactaaaaatacaaaaaattagccgggcgtggtggcgggcgcctgtagtcccagctactcgggaggctgaggcaggagaatggcgtgaacccgggaggcggagcttgcagtgagccgagatcacgccgctgcactccaccctgggcgacagagcgagactccgtctcaaaaaaaaaaaaaaaaaaaaaaaaaaaaaagattaataactgctggagatccaagagcgagccaacagatttttttttaattttaattttaattttaattttaattttaaacgcgtcgacgtcggccatagcggccgcggaa

SEQ ID NO: 18 - DNA, 18 bp, Artificial sequence
  The upstream primer sequence for detecting the inserted sequence in example 3.
tttcagggtctaggtggc

SEQ ID NO: 19 - DNA, 18 bp, Artificial sequence
  The downstream primer sequence for detecting the inserted sequence in example 3.
aaatgctttctccgctct

SEQ ID NO: 20 - DNA, 20 bp, Artificial sequence
  The upstream primer sequence for detecting the connection in example 4.
ggcataatgatgtggctgtt

SEQ ID NO: 21 - DNA, 18 bp, Artificial sequence
  The downstream primer sequence for detecting the connection in example 4.
tctgttggctcgctcttg

SEQ ID NO: 22 - DNA, 606 bp, Artificial sequence
  The Seq ID No.15 with 6bp sequence in the upstream sequence of target site replaced with “CGATGA”.
ctagctagctagagcatggcgatggatacccctttgacggtaaggacggactcctggctcatgccttcgccccaggcactggtgttgggggagactcccattttgatgacgatgagctatggaccttgggagaaggccaaggtgagaaaggggccctctgcatgccccagaccttctctcctgtcctctctccactccatttgcttgcgatgaagagcctgtgggccttgctcagagcggagaaagcatggcataatgatgtggctgttttgtttgtacaagatccgcagacgtgtaaatgttcctgcaaaaacacagacgtgggaggggaggaaagtcacacatctgggtgagtcagaatcttggtctccaaagaaggcctggagaagtccaacctcccccttccatgtcactctttagtggtccgtgtgaagtatgggaacgccgatggggagtactgcaagttccccttcttgttcaatggcaaggagtacaacagctgcactgataccggccgcagcgatggcttcctctggtgctccaccacctacaactttgagaaggatggcaagtacggcttctgtccccatgaagctagctagctag

SEQ ID NO: 23 - DNA, 160 bp, Artificial sequence
  The 160bp selected sequence of gene IT15 in the human genome.
atgctattcataatcacattcgtttgtttgaacctcttgttataaaagctttaaaacagtacacgactacaacatgtgtgcagttacagaagcaggttttagatttgctggcgcagctggttcagttacgggttaattactgtcttctggattcagatca

SEQ ID NO: 24 - DNA, 461 bp, Artificial sequence
  The Seq ID No.23 with the sequence to be inserted, partial Alu sequence, NheI enzyme cutting sites and protective bases.
ctagctagctagatgctattcataatcacattcgtttgtttgaacctcttgttataaaagctttaaaacagtacacgactacaacatgtgtgcagttacaggaagttcatggatgtctatcagcgcagctactgccatccaatcgagaccctggtggacataagcaggttttagatttgctggcgcagctggttcagttacgggttaattactgtcttctggattcagatcaactaaaaatacaaaaaattagccgggcgtggtggcgggcgcctgtagtcccagctactcgggaggctgaggcaggagaatggcgtgaacccgggaggcggagcttgcagtgagccgagatcacgccgctgcactccaccctgggcgacagagcgagactccgtctcaaaaaaaaaaaaaaaaaaaaaaaaaaaaaagattaataactgctggagatcctagctagctag

SEQ ID NO: 25 - DNA, 20 bp, Artificial sequence
  The upstream primer sequence for detecting the inserted sequence in example 6.
gaaattggtttgagcaggag

SEQ ID NO: 26 - DNA, 18 bp, Artificial sequence
  The downstream primer sequence for detecting the inserted sequence in example 6.
cgattggatggcagtagc

SEQ ID NO: 27 - DNA, 461 bp, Artificial sequence
  The Seq ID No.24 with 6bp sequence in the upstream sequence of target site replaced with “GGACAT”.
ctagctagctagatgctattcataatcacattcgtttgtttgaacctcttgttataaaagctttaaaacagtacacgactacaacaggacatcagttacaggaagttcatggatgtctatcagcgcagctactgccatccaatcgagaccctggtggacataagcaggttttagatttgctggcgcagctggttcagttacgggttaattactgtcttctggattcagatcaactaaaaatacaaaaaattagccgggcgtggtggcgggcgcctgtagtcccagctactcgggaggctgaggcaggagaatggcgtgaacccgggaggcggagcttgcagtgagccgagatcacgccgctgcactccaccctgggcgacagagcgagactccgtctcaaaaaaaaaaaaaaaaaaaaaaaaaaaaaagattaataactgctggagatcctagctagctag

SEQ ID NO: 28 - DNA, 1148 bp, Artificial sequence
  The selected sequence of gene MINK1 in the human genome.
agagaatgaggggcccctttttctctctggtggctcaggcccaactcccttcctactggggaggctcactccctcccctttcccctctccccctggaatgccctgcctcctgctgaaaatccctcaggaagctcttcacctgtcacctgttacgggccaggtgctctgcaggttgctctggggagatgggatctgatggccctcctgcctgggatgctgtccgtgatccttttacctgggtttttctctaagatgctggaagatggaatcgggttcttcaggatggtggtggggtaaaggagggtgctggggtgtctgggtcgggccaggaccacagctggctcaggcaagtcctgtgtgtgcacgcagggatgtgaggcaagggagcagaggtgactccccacactgacccctccctctgtgtcttcacagtggattttggggtgagtgctcagctggaccgcaccgtgggcagacggaacactttcattgggactccctactggatggctccagaggtcatcgcctgtgatgagaaccctgatgccacctatgattacagggtatggagtggaaagttgggagcatgggggctgccaagggcgggaagcaatatggggaccacggggcctgagcaggctggggaacagaggaaggtcagatgatgttagcagtgaggggctggggaacatcttacggcaaggcaagtgtgggtgggaagatgggatgggttggaaggcactgctgcaggaatgggtgtggcccaggaaggctcctgagaggccaggatggtgggtgaagagaggttgcagggcagagttgtcaggaatattcacttgttccttctttcccgtctatagagtgatatttggtctctaggaatcacagccatcgagatggcagagggagccccccgtaagttctgagtctgccgggagtgggaggggagggaaaggaagggcccagagagtggctgtagggaggaggtgggtcctgggaccctgccgaggaagggtcctgtagctcccagtgcagtgaaagggactgagggtgtctcctctgtgtccagctctgtgtgacatgcaccccatgcgagccctcttcctcattcctcggaaccctccgcccaggctcaagtccaagaagtg

SEQ ID NO: 29 - DNA, 492 bp, Artificial sequence
  The sequence used in the deletion based on the Seq ID No.28.
ctagctagctagagtgatatttggtctctaggaatcacagccatcgagatggcagagggagccccccgtaagttctgagtctgccagagaatgaggggcccctttttctctctggtggctcaggcccaactcccttcctactggggaggctcactccctcccctttcccctctccccctggaatgccctgcctcctgctgaaaatccctcaggaagctcttcacctgtcacctgttacgggccaggtgctctgcaggttgctctggggagtgggaggggagggaaaggaagggcccagagagtggctgtagggaggaggtgggtcctgggaccctgccgaggaagggtcctgtagctcccagtgcagtgaaagggactgagggtgtctcctctgtgtccagctctgtgtgacatgcaccccatgcgagccctcttcctcattcctcggaaccctccgcccaggctcaagtccaagaagtgctagctagctag

SEQ ID NO: 30 - DNA, 492 bp, Artificial sequence
  The Seq ID No.29 with a sequence that is not homologous to the MINK1 gene replacing the upstream sequence immediately adjacent to the 5′ end of the sequence to be deleted in Seq ID No. 29.
ctagctagctagagtgatatttggtctctaggaatcacagccatcgagatggcagagggagccccccgtaagttctgagtctgcccattgttataatgattaaacaagttatatatgaaaagattaaaacagtgttgctccataataaatgctgtttttactgtgattattattgttgttatccctatcattatcatcaccatcttaacccttccctgttttgctcttttctctctccctacccattgcagaccaaagaaagatagggagtgggaggggagggaaaggaagggcccagagagtggctgtagggaggaggtgggtcctgggaccctgccgaggaagggtcctgtagctcccagtgcagtgaaagggactgagggtgtctcctctgtgtccagctctgtgtgacatgcaccccatgcgagccctcttcctcattcctcggaaccctccgcccaggctcaagtccaagaagtgctagctagctag

SEQ ID NO: 31 - DNA, 20 bp, Artificial sequence
  The upstream primer sequence for detecting the deletion in example 8.
acagggtatggagtggaaag

SEQ ID NO: 32 - DNA, 20 bp, Artificial sequence
  The downstream primer sequence for detecting the deletion in example 8.
atagacgggaaagaaggaac

SEQ ID NO: 33 - DNA, 806 bp, Artificial sequence
  The selected sequence of gene FMR1 in the human genome.
acttgctgagtacccaaggaaagtgtgcttgtatttatgggcgtctattttcagagcactaattattgctgaattagaacagaaatataggaaaactgatttttacaaggagcttcaaagcaatctcaggtagtttctgattatgtatctctgcctacctcggggtacatagacagggttacaatttggttgaggatatatgacatgtggtttttaaagacacctaggggcattttaagaaaatttcctcgatatctgaaaatctgtagatttcaaaattatgttaatcatgaaatattctgtgttgtaatttttgtgtaggtgtattccagagcaaatgaaaaagagccttgctgttggtggttagctaaagtgaggatgataaagggtgaggtaggaaaatgcctatttaaatttttttcttatattgtttcctttttttaaacccaggttgtacattcccgtgtggatttctattttgaagtaatatctaattttgagtaatttaattaaaatgttttcactatgtgttcagtatgtttctgttggtcataaattttttcacatagattatttattttaaaataactgaatagggagaacttcttattcttactttaaaaattgtgattagaagtgacttttatttatttctcagttttatgtgatagaatatgcagcatgtgatgcaacttacaatgaaattgtcacaattgaacgtctaagatctgttaatcccaacaaacctgccacaaaagatactttccataagatcaagctggatgtgccagaagacttacggcaaa

SEQ ID NO: 34 - DNA, 488 bp, Artificial sequence
  The sequence used in the deletion based on the Seq ID No.33.
ctagctagctagtttatgtgatagaatatgcagcatgtgatgcaacttacaatgaaattgtcacaattgaacgtctaagatctgttaatcccaacaaacctgccacaaaagacttgctgagtacccaaggaaagtgtgcttgtatttatgggcgtctattttcagagcactaattattgctgaattagaacagaaatataggaaaactgatatactttccataagatcaagctggatgtgccagaagacttacggcaaaactaaaaatacaaaaaattagccgggcgtggtggcgggcgcctgtagtcccagctactcgggaggctgaggcaggagaatggcgtgaacccgggaggcggagcttgcagtgagccgagatcacgccgctgcactccaccctgggcgacagagcgagactccgtctcaaaaaaaaaaaaaaaaaaaaaaaaaaaaaagattaataactgctggagatcctagctagctag

SEQ ID NO: 35 - DNA, 488 bp, Artificial sequence
  The Seq ID No.34 with a sequence that is not homologous to the MINK1 gene replacing the upstream sequence immediately adjacent to the 5′ end of the sequence to be deleted in Seq ID No. 34.
ctagctagctagtttatgtgatagaatatgcagcatgtgatgcaacttacaatgaaattgtcacaattgaacgtctaagatctgttaatcccaacaaacctgccacaaaagagtgttgctccataataaatgctgtttttactgtgattattattgttgttatccctatcattatcatcaccatcttaacccttccctgttttgctcttttatactttccataagatcaagctggatgtgccagaagacttacggcaaaactaaaaatacaaaaaattagccgggcgtggtggcgggcgcctgtagtcccagctactcgggaggctgaggcaggagaatggcgtgaacccgggaggcggagcttgcagtgagccgagatcacgccgctgcactccaccctgggcgacagagcgagactccgtctcaaaaaaaaaaaaaaaaaaaaaaaaaaaaaagattaataactgctggagatcctagctagctag

SEQ ID NO: 36 - DNA, 18 bp, Artificial sequence
  The upstream primer sequence for detecting the deletion in example 9.
acagggttacaatttggt

SEQ ID NO: 37 - DNA, 19 bp, Artificial sequence
  The downstream primer sequence for detecting the deletion in example 9.
catttgctctggaatacac

SEQ ID NO: 38 - DNA, 461 bp, Artificial sequence
  The gene transcription framework designed based on IT15 gene and partial Alu sequence, with NheI digestion recognition site and protection bases at both ends.
ctagctagctagatgctattcataatcacattcgtttgtttgaacctcttgttataaaagctttaaaacagtacacgactacgaagttcatggatgtctatcagcgcagctactgccatccaatcgagaccctggtggacataacatgtgtgcagttacagaagcaggttttagatttgctggcgcagctggttcagttacgggttaattactgtcttctggattcagatcaactaaaaatacaaaaaattagccgggcgtggtggcgggcgcctgtagtcccagctactcgggaggctgaggcaggagaatggcgtgaacccgggaggcggagcttgcagtgagccgagatcacgccgctgcactccaccctgggcgacagagcgagactccgtctcaaaaaaaaaaaaaaaaaaaaaaaaaaaaaagattaataactgctggagatcctagctagctag

SEQ ID NO: 39 - DNA, 1425 bp, Artificial sequence
  The 3′ sequence of the BRCA1 gene selected intron.
cccagctacttgagaggctgaggcagggagaattgcttgaaccaggtaggcggaggttgcagtgagccaagatcgcaccactgcactccagcctggggcaacagagcaagactgtctcaaaaaaaataaataaataaaataaattcttaagaaggatattttggaaaactccttacatacctaaattctttgtttatcaaatacttggacttagcacactcttctttgaaatggaccaataaacaacaggagcccataagcaaaaagaactcattattttaaaaacagtaactatccttacaggctttctcagggctctttctgttggatccttccctctcacaggtccttgctaatgatctctaggtggacacattctagatgagatgtccctgtctagaatggcagcaccatgagggctatatcctcagtactaggacagcgcctggtgcttaatagatagtaaatagttgtctaattaactgagcaaacagatagattcatgaattagctttttgctttttctgttagaaactaaaggttcaggtcaggcacaatggcgcatgtctctaatcccagcactttgggaggccgaggcgggctgatcacttgaggtcaggagttcaagaccagcctggccaacatagtaaaaccctgtttctacaaaaattaccaaaattagccgggcgtcttggcaagcacctgtaatgccagctacttgagaggctgaggtgggagaatcgcttgaacctgggaggaagaggttgcagtgagccgagatggtgccaacctgggtgacagagggagacttaaaaaaaaaaagaaagaaagaaagaaaagaaactaaaggttcaaagaatcccagaaaaggaagagtcctcacaagccagtaatctaggcaggattactgatagtatttttatatttgttgtatttttataaaatgccatagatagagggcttttttcaacattacatcagtctaaaaatcacacatttttatatgaactaacctaaatgtctgatgaatctcacaacaccaagtctttgaaatgtgcccatataaataaaatgttaacagattcatgctaattttaaatatcgatagtgtttaaatgccttaattattttttcactccctagctttaaaagaaaataaccaacttcaaaaggacatcacaataacatcaagtctatttgggggaatttgaggattttttccctcactaacatcatttggaaataatttcatgggcattaattgcatgaatgtggttagattaaaaggtgttcagctagaacttgtagttccatactaggtgatttcaattcctgtgctaaaattaatttgtatgatatattttcatttaatggaaagcttctcaaagtatttcattttcttggtgccatttatcgtttttgaag

SEQ ID NO: 40 - DNA, 421 bp, Artificial sequence
  The 3′ end sequence of the sequence to be deleted (Example 11) + the randomly designed sequence that is not homologous to the BRCA 1 gene + partial Alu sequence (Possible natural shear site versio n 1), with NheI digestion site and protective bases at both ends.
ctagctagctagactaacatcatttggaaataatttcatgggcattaattgcatgaatgtggttagattaaaaggtgttcagctagaacttgtagttccatactaggtgatttcaattcctgtgctaaaattaatttgtatgatatattttcatttaatggaaagcttctcaaagtatttcattttcttggtgccatttatcgtttttgaagggggggaaaaatacaaaaaattagccgggcgtgatggtgggcgcctgtagtcccagctacacgggaggctgagacaggagaatggcgtgaacccgggaggcggagcttgcagtgagccgagatcgcaccactgcactgcagcctgggcgacagagcgagactctgtctcaaaaaaaaaaaaaaagaaagaaaaaaaactagctagctag

SEQ ID NO: 41 - DNA, 423 bp, Artificial sequence
  The 3′ end sequence of the sequence to be deleted (Example 11) + the randomly designed sequence that is not homologous to the BRCA 1 gene + partial Alu sequence (Possible natural shear site versio n 2), with NheI digestion site and protective bases at both ends.
ctagctagctagactaacatcatttggaaataatttcatgggcattaattgcatgaatgtggttagattaaaaggtgttcagctagaacttgtagttccatactaggtgatttcaattcctgtgctaaaattaatttgtatgatatattttcatttaatggaaagcttctcaaagtatttcattttcttggtgccatttatcgtttttgaagggggggctaaaaatacaaaaaattagccgggcgtgatggtgggcgcctgtagtcccagctacacgggaggctgagacaggagaatggcgtgaacccgggaggcggagcttgcagtgagccgagatcgcaccactgcactgcagcctgggcgacagagcgagactctgtctcaaaaaaaaaaaaaaagaaagaaaaaaaactagctagctag

SEQ ID NO: 42 - DNA, 424 bp, Artificial sequence
  The 3′ end sequence of the sequence to be deleted (Example 11) + the randomly designed sequence that is not homologous to the BRCA 1 gene + partial Alu sequence (Possible natural shear site versio n 3), with NheI digestion site and protective bases at both ends.
ctagctagctagactaacatcatttggaaataatttcatgggcattaattgcatgaatgtggttagattaaaaggtgttcagctagaacttgtagttccatactaggtgatttcaattcctgtgctaaaattaatttgtatgatatattttcatttaatggaaagcttctcaaagtatttcattttcttggtgccatttatcgtttttgaagggggggactaaaaatacaaaaaattagccgggcgtgatggtgggcgcctgtagtcccagctacacgggaggctgagacaggagaatggcgtgaacccgggaggcggagcttgcagtgagccgagatcgcaccactgcactgcagcctgggcgacagagcgagactctgtctcaaaaaaaaaaaaaaagaaagaaaaaaaactagctagctag

SEQ ID NO: 43 - DNA, 415 bp, Artificial sequence
  The Seq ID No.40 without non-homologous sequences.
ctagctagctagactaacatcatttggaaataatttcatgggcattaattgcatgaatgtggttagattaaaaggtgttcagctagaacttgtagttccatactaggtgatttcaattcctgtgctaaaattaatttgtatgatatattttcatttaatggaaagcttctcaaagtatttcattttcttggtgccatttatcgtttttgaagaaaaatacaaaaaattagccgggcgtgatggtgggcgcctgtagtcccagctacacgggaggctgagacaggagaatggcgtgaacccgggaggcggagcttgcagtgagccgagatcgcaccactgcactgcagcctgggcgacagagcgagactctgtctcaaaaaaaaaaaaaaagaaagaaaaaaaactagctagctag

SEQ ID NO: 44 - DNA, 417 bp, Artificial sequence
  The Seq ID No.41 without non-homologous sequences.
ctagctagctagactaacatcatttggaaataatttcatgggcattaattgcatgaatgtggttagattaaaaggtgttcagctagaacttgtagttccatactaggtgatttcaattcctgtgctaaaattaatttgtatgatatattttcatttaatggaaagcttctcaaagtatttcattttcttggtgccatttatcgtttttgaagctaaaaatacaaaaaattagccgggcgtgatggtgggcgcctgtagtcccagctacacgggaggctgagacaggagaatggcgtgaacccgggaggcggagcttgcagtgagccgagatcgcaccactgcactgcagcctgggcgacagagcgagactctgtctcaaaaaaaaaaaaaaagaaagaaaaaaaactagctagctag

SEQ ID NO: 45 - DNA, 418 bp, Artificial sequence
  The Seq ID No.42 without non-homologous sequences.
ctagctagctagactaacatcatttggaaataatttcatgggcattaattgcatgaatgtggttagattaaaaggtgttcagctagaacttgtagttccatactaggtgatttcaattcctgtgctaaaattaatttgtatgatatattttcatttaatggaaagcttctcaaagtatttcattttcttggtgccatttatcgtttttgaagactaaaaatacaaaaaattagccgggcgtgatggtgggcgcctgtagtcccagctacacgggaggctgagacaggagaatggcgtgaacccgggaggcggagcttgcagtgagccgagatcgcaccactgcactgcagcctgggcgacagagcgagactctgtctcaaaaaaaaaaaaaaagaaagaaaaaaaactagctagctag

SEQ ID NO: 46 - DNA, 18 bp, Artificial sequence
  The upstream primer sequence for detecting the downstream sequence of the 3′ end sequence of the sequence to be deleted in example 11.
cccctttatctccttctg

SEQ ID NO: 47 - DNA, 18 bp, Artificial sequence
  The downstream primer sequence for detecting the downstream sequence of the 3′ end sequence of the sequence to be deleted in example 11.
atttctcccattccactt

SEQ ID NO: 48 - DNA, 571 bp, Artificial sequence
  The 3′ end sequence of the sequence to be deleted (Example 12) + non-homologous sequence + upstream sequence immediately adjacent to the 5′ end of the sequence to be deleted + partial Alu sequenc e (Possible natural shear site version 1), with NheI digestion si
ctagctagctagactaacatcatttggaaataatttcatgggcattaattgcatgaatgtggttagattaaaaggtgttcagctagaacttgtagttccatactaggtgatttcaattcctgtgctaaaattaatttgtatgatatattttcatttaatggaaagcttctcaaagtatttcattttcttggtgccatttatcgtttttgaagggggggcccagctacttgagaggctgaggcagggagaattgcttgaaccaggtaggcggaggttgcagtgagccaagatcgcaccactgcactccagcctggggcaacagagcaagactgtctcaaaaaaaataaataaataaaataaattcttaaaaaaatacaaaaaattagccgggcgtgatggtgggcgcctgtagtcccagctacacgggaggctgagacaggagaatggcgtgaacccgggaggcggagcttgcagtgagccgagatcgcaccactgcactgcagcctgggcgacagagcgagactctgtctcaaaaaaaaaaaaaaagaaagaaaaaaaactagctagctag

SEQ ID NO: 49 - DNA, 573 bp, Artificial sequence
  The 3′ end sequence of the sequence to be deleted (Example 12) + non-homologous sequence + upstream sequence immediately adjacent to the 5′ end of the sequence to be deleted + partial Alu sequenc e (Possible natural shear site version 2), with NheI digestion si
ctagctagctagactaacatcatttggaaataatttcatgggcattaattgcatgaatgtggttagattaaaaggtgttcagctagaacttgtagttccatactaggtgatttcaattcctgtgctaaaattaatttgtatgatatattttcatttaatggaaagcttctcaaagtatttcattttcttggtgccatttatcgtttttgaagggggggcccagctacttgagaggctgaggcagggagaattgcttgaaccaggtaggcggaggttgcagtgagccaagatcgcaccactgcactccagcctggggcaacagagcaagactgtctcaaaaaaaataaataaataaaataaattcttaactaaaaatacaaaaaattagccgggcgtgatggtgggcgcctgtagtcccagctacacgggaggctgagacaggagaatggcgtgaacccgggaggcggagcttgcagtgagccgagatcgcaccactgcactgcagcctgggcgacagagcgagactctgtctcaaaaaaaaaaaaaaagaaagaaaaaaaactagctagctag

SEQ ID NO: 50 - DNA, 574 bp, Artificial sequence
  The 3′ end sequence of the sequence to be deleted (Example 12) + non-homologous sequence + upstream sequence immediately adjacent to the 5′ end of the sequence to be deleted + partial Alu sequenc e (Possible natural shear site version 3), with NheI digestion si
ctagctagctagactaacatcatttggaaataatttcatgggcattaattgcatgaatgtggttagattaaaaggtgttcagctagaacttgtagttccatactaggtgatttcaattcctgtgctaaaattaatttgtatgatatattttcatttaatggaaagcttctcaaagtatttcattttcttggtgccatttatcgtttttgaagggggggcccagctacttgagaggctgaggcagggagaattgcttgaaccaggtaggcggaggttgcagtgagccaagatcgcaccactgcactccagcctggggcaacagagcaagactgtctcaaaaaaaataaataaataaaataaattcttaaactaaaaatacaaaaaattagccgggcgtgatggtgggcgcctgtagtcccagctacacgggaggctgagacaggagaatggcgtgaacccgggaggcggagcttgcagtgagccgagatcgcaccactgcactgcagcctgggcgacagagcgagactctgtctcaaaaaaaaaaaaaaagaaagaaaaaaaactagctagctag

SEQ ID NO: 51 - DNA, 18 bp, Artificial sequence
  The upstream primer sequence for detecting the deletion in example 12.
gctttctcagggctcttt

SEQ ID NO: 52 - DNA, 18 bp, Artificial sequence
  The downstream primer sequence for detecting the deletion in example 12.
gcaccatctcggctcact

SEQ ID NO: 53 - DNA, 21 bp, Artificial sequence
  The upstream primer sequence for detecting the expression of BRCA1 in example 13.
cagaggacaatggcttccatg

SEQ ID NO: 54 - DNA, 24 bp, Artificial sequence
  The downstream primer sequence for detecting the expression of BRCA1 in example 13.
ctacactgtccaacacccactctc